European Patent Application EP 4 470 615 A2, published December 4, 2024. Title: SMALL RNA MEDICAMENT FOR PREVENTION AND TREATMENT OF INFLAMMATION-RELATED DISEASES AND COMBINATION THEREOF. Applicant: INSTITUTE OF BASIC MEDICAL SCIENCES CHINESE ACADEMY OF MEDICAL SCIENCES. Application EP 18944638.8, filed December 25, 2018. The sequence listing filed with the application follows.

SEQUENCE LISTING (239 sequences)

SEQ ID NO: 1 - RNA, 18 nt, synthetic construct
  misc_feature 1..18: note = BZL-sRNA-1
  source 1..18: mol_type = other RNA
gttcagagttctacagtc

SEQ ID NO: 2 - RNA, 21 nt, synthetic construct
  misc_feature 1..21: note = BZL-sRNA-2
  source 1..21: mol_type = other RNA
gttcagagttctacagtccga

SEQ ID NO: 3 - RNA, 24 nt, synthetic construct
  misc_feature 1..24: note = BZL-sRNA-3
  source 1..24: mol_type = other RNA
tcagagttctacagtccgacgatc

SEQ ID NO: 4 - RNA, 24 nt, synthetic construct
  misc_feature 1..24: note = BZL-sRNA-4
  source 1..24: mol_type = other RNA
gttcagagttctacagtccgacga

SEQ ID NO: 5 - RNA, 20 nt, synthetic construct
  misc_feature 1..20: note = BZL-sRNA-5
  source 1..20: mol_type = other RNA
tcagtctttttctctctcct

SEQ ID NO: 6 - RNA, 26 nt, synthetic construct
  misc_feature 1..26: note = BZL-sRNA-6
  source 1..26: mol_type = other RNA
tctcgcttggggtgcgagaggtcccg

SEQ ID NO: 7 - RNA, 21 nt, synthetic construct
  misc_feature 1..21: note = BZL-sRNA-7
  source 1..21: mol_type = other RNA
tcagtctttttctctctccta

SEQ ID NO: 8 - RNA, 19 nt, synthetic construct
  misc_feature 1..19: note = BZL-sRNA-8
  source 1..19: mol_type = other RNA
tccggtatggtctagtggc

SEQ ID NO: 9 - RNA, 20 nt, synthetic construct
  misc_feature 1..20: note = BZL-sRNA-9
  source 1..20: mol_type = other RNA
taggaacttcataccgtgct

SEQ ID NO: 10 - RNA, 22 nt, synthetic construct
  misc_feature 1..22: note = BZL-sRNA-10
  source 1..22: mol_type = other RNA
tcagtctttttctctctcctat

SEQ ID NO: 11 - RNA, 21 nt, synthetic construct
  misc_feature 1..21: note = BZL-sRNA-11
  source 1..21: mol_type = other RNA
taggaacttcataccgtgctc

SEQ ID NO: 12 - RNA, 22 nt, synthetic construct
  misc_feature 1..22: note = BZL-sRNA-12
  source 1..22: mol_type = other RNA
taggaacttcataccgtgctct

SEQ ID NO: 13 - RNA, 22 nt, synthetic construct
  misc_feature 1..22: note = BZL-sRNA-13
  source 1..22: mol_type = other RNA
tggaatgtaaagaagtatggag

SEQ ID NO: 14 - RNA, 21 nt, synthetic construct
  misc_feature 1..21: note = BZL-sRNA-14
  source 1..21: mol_type = other RNA
tgaacacagctggtggtatct

SEQ ID NO: 15 - RNA, 20 nt, synthetic construct
  misc_feature 1..20: note = BZL-sRNA-15
  source 1..20: mol_type = other RNA
gggggcgtagctcagatggt

SEQ ID NO: 16 - RNA, 20 nt, synthetic construct
  misc_feature 1..20: note = BZL-sRNA-16
  source 1..20: mol_type = other RNA
ggatttgagtaagagcgtag

SEQ ID NO: 17 - RNA, 21 nt, synthetic construct
  misc_feature 1..21: note = BZL-sRNA-17
  source 1..21: mol_type = other RNA
tggatttgagtaagagcgtag

SEQ ID NO: 18 - RNA, 22 nt, synthetic construct
  misc_feature 1..22: note = BZL-sRNA-18
  source 1..22: mol_type = other RNA
atggatttgagtaagagcgtag

SEQ ID NO: 19 - RNA, 25 nt, synthetic construct
  misc_feature 1..25: note = BZL-sRNA-19
  source 1..25: mol_type = other RNA
gttcagagttctacagtccgacgat

SEQ ID NO: 20 - RNA, 26 nt, synthetic construct
  misc_feature 1..26: note = BZL-sRNA-20
  source 1..26: mol_type = other RNA
gttcagagttctacagtccgacgatc

SEQ ID NO: 21 - RNA, 23 nt, synthetic construct
  misc_feature 1..23: note = BZL-sRNA-21
  source 1..23: mol_type = other RNA
gatggatttgagtaagagcgtag

SEQ ID NO: 22 - RNA, 18 nt, synthetic construct
  misc_feature 1..18: note = BZL-sRNA-22
  source 1..18: mol_type = other RNA
ctcttcaacgaggaatgc

SEQ ID NO: 23 - RNA, 24 nt, synthetic construct
  misc_feature 1..24: note = BZL-sRNA-23
  source 1..24: mol_type = other RNA
ggatggatttgagtaagagcgtag

SEQ ID NO: 24 - RNA, 18 nt, synthetic construct
  misc_feature 1..18: note = BZL-sRNA-24
  source 1..18: mol_type = other RNA
gaaacggctgctaatacc

SEQ ID NO: 25 - RNA, 20 nt, synthetic construct
  misc_feature 1..20: note = BZL-sRNA-25
  source 1..20: mol_type = other RNA
tggaaacggctgctaatacc

SEQ ID NO: 26 - RNA, 21 nt, synthetic construct
  misc_feature 1..21: note = BZL-sRNA-26
  source 1..21: mol_type = other RNA
tggatttgagtaagagcatag

SEQ ID NO: 27 - RNA, 22 nt, synthetic construct
  misc_feature 1..22: note = BZL-sRNA-27
  source 1..22: mol_type = other RNA
atggatttgagtaagagcatag

SEQ ID NO: 28 - RNA, 18 nt, synthetic construct
  misc_feature 1..18: note = BZL-sRNA-28
  source 1..18: mol_type = other RNA
ccccgtcgtgcccggacc

SEQ ID NO: 29 - RNA, 25 nt, synthetic construct
  misc_feature 1..25: note = BZL-sRNA-29
  source 1..25: mol_type = other RNA
cggatggatttgagtaagagcgtag

SEQ ID NO: 30 - RNA, 21 nt, synthetic construct
  misc_feature 1..21: note = BZL-sRNA-30
  source 1..21: mol_type = other RNA
ctggaaacggctgctaatacc

SEQ ID NO: 31 - RNA, 19 nt, synthetic construct
  misc_feature 1..19: note = BZL-sRNA-31
  source 1..19: mol_type = other RNA
gccccgtcgtgcccggacc

SEQ ID NO: 32 - RNA, 23 nt, synthetic construct
  misc_feature 1..23: note = BZL-sRNA-32
  source 1..23: mol_type = other RNA
agctggaaacggctgctaatacc

SEQ ID NO: 33 - RNA, 20 nt, synthetic construct
  misc_feature 1..20: note = BZL-sRNA-33
  source 1..20: mol_type = other RNA
agccccgtcgtgcccggacc

SEQ ID NO: 34 - RNA, 21 nt, synthetic construct
  misc_feature 1..21: note = BZL-sRNA-34
  source 1..21: mol_type = other RNA
gagccccgtcgtgcccggacc

SEQ ID NO: 35 - RNA, 22 nt, synthetic construct
  misc_feature 1..22: note = BZL-sRNA-35
  source 1..22: mol_type = other RNA
agagccccgtcgtgcccggacc

SEQ ID NO: 36 - RNA, 23 nt, synthetic construct
  misc_feature 1..23: note = BZL-sRNA-36
  source 1..23: mol_type = other RNA
gagagccccgtcgtgcccggacc

SEQ ID NO: 37 - RNA, 24 nt, synthetic construct
  misc_feature 1..24: note = BZL-sRNA-37
  source 1..24: mol_type = other RNA
tgagagccccgtcgtgcccggacc

SEQ ID NO: 38 - RNA, 25 nt, synthetic construct
  misc_feature 1..25: note = BZL-sRNA-38
  source 1..25: mol_type = other RNA
gtgagagccccgtcgtgcccggacc

SEQ ID NO: 39 - RNA, 26 nt, synthetic construct
  misc_feature 1..26: note = BZL-sRNA-39
  source 1..26: mol_type = other RNA
ggtgagagccccgtcgtgcccggacc

SEQ ID NO: 40 - RNA, 27 nt, synthetic construct
  misc_feature 1..27: note = BZL-sRNA-40
  source 1..27: mol_type = other RNA
gggtgagagccccgtcgtgcccggacc

SEQ ID NO: 41 - RNA, 28 nt, synthetic construct
  misc_feature 1..28: note = BZL-sRNA-41
  source 1..28: mol_type = other RNA
agggtgagagccccgtcgtgcccggacc

SEQ ID NO: 42 - RNA, 29 nt, synthetic construct
  misc_feature 1..29: note = BZL-sRNA-42
  source 1..29: mol_type = other RNA
gagggtgagagccccgtcgtgcccggacc

SEQ ID NO: 43 - RNA, 18 nt, synthetic construct
  misc_feature 1..18: note = CHu-sRNA-1
  source 1..18: mol_type = other RNA
acaactttcagcaacgga

SEQ ID NO: 44 - RNA, 19 nt, synthetic construct
  misc_feature 1..19: note = CHu-sRNA-2
  source 1..19: mol_type = other RNA
acaactttcagcaacggat

SEQ ID NO: 45 - RNA, 20 nt, synthetic construct
  misc_feature 1..20: note = CHu-sRNA-3
  source 1..20: mol_type = other RNA
acaactttcagcaacggatc

SEQ ID NO: 46 - RNA, 21 nt, synthetic construct
  misc_feature 1..21: note = CHu-sRNA-4
  source 1..21: mol_type = other RNA
acaactttcagcaacggatct

SEQ ID NO: 47 - RNA, 20 nt, synthetic construct
  misc_feature 1..20: note = CHu-sRNA-5
  source 1..20: mol_type = other RNA
tgatatgaagcactgtagct

SEQ ID NO: 48 - RNA, 21 nt, synthetic construct
  misc_feature 1..21: note = CHu-sRNA-6
  source 1..21: mol_type = other RNA
tgatatgaagcactgtagctc

SEQ ID NO: 49 - RNA, 19 nt, synthetic construct
  misc_feature 1..19: note = CHu-sRNA-7
  source 1..19: mol_type = other RNA
gttcagagttctacagtcc

SEQ ID NO: 50 - RNA, 20 nt, synthetic construct
  misc_feature 1..20: note = CHu-sRNA-8
  source 1..20: mol_type = other RNA
gttcagagttctacagtccg

SEQ ID NO: 51 - RNA, 19 nt, synthetic construct
  misc_feature 1..19: note = CHu-sRNA-9
  source 1..19: mol_type = other RNA
tgtagtagattgtatagtt

SEQ ID NO: 52 - RNA, 22 nt, synthetic construct
  misc_feature 1..22: note = CHu-sRNA-10
  source 1..22: mol_type = other RNA
tgatatgaagcactgtagctct

SEQ ID NO: 53 - RNA, 18 nt, synthetic construct
  misc_feature 1..18: note = CHu-sRNA-11
  source 1..18: mol_type = other RNA
tgatgtagtaggttgtat

SEQ ID NO: 54 - RNA, 19 nt, synthetic construct
  misc_feature 1..19: note = CHu-sRNA-12
  source 1..19: mol_type = other RNA
tgatgtagtagattgtata

SEQ ID NO: 55 - RNA, 20 nt, synthetic construct
  misc_feature 1..20: note = CHu-sRNA-13
  source 1..20: mol_type = other RNA
tgatgtagtagattgtatag

SEQ ID NO: 56 - RNA, 21 nt, synthetic construct
  misc_feature 1..21: note = CHu-sRNA-14
  source 1..21: mol_type = other RNA
tgatgtagtagattgtatagt

SEQ ID NO: 57 - RNA, 22 nt, synthetic construct
  misc_feature 1..22: note = CHu-sRNA-15
  source 1..22: mol_type = other RNA
tgatgtagtagattgtatagtt

SEQ ID NO: 58 - RNA, 18 nt, synthetic construct
  misc_feature 1..18: note = CHu-sRNA-16
  source 1..18: mol_type = other RNA
tgctgtagtaggttgtat

SEQ ID NO: 59 - RNA, 20 nt, synthetic construct
  misc_feature 1..20: note = CHu-sRNA-17
  source 1..20: mol_type = other RNA
tgatgtagtaggttgtatgg

SEQ ID NO: 60 - RNA, 21 nt, synthetic construct
  misc_feature 1..21: note = CHu-sRNA-18
  source 1..21: mol_type = other RNA
tgatgtagtaggttgtatggt

SEQ ID NO: 61 - RNA, 20 nt, synthetic construct
  misc_feature 1..20: note = CHu-sRNA-19
  source 1..20: mol_type = other RNA
tgatgtagtaggttgtatag

SEQ ID NO: 62 - RNA, 18 nt, synthetic construct
  misc_feature 1..18: note = CHu-sRNA-20
  source 1..18: mol_type = other RNA
agccggacggtggccatg

SEQ ID NO: 63 - RNA, 21 nt, synthetic construct
  misc_feature 1..21: note = CHu-sRNA-21
  source 1..21: mol_type = other RNA
taacttatcagactgatgttg

SEQ ID NO: 64 - RNA, 22 nt, synthetic construct
  misc_feature 1..22: note = CHu-sRNA-22
  source 1..22: mol_type = other RNA
cagcagcaattcatgttttgga

SEQ ID NO: 65 - RNA, 22 nt, synthetic construct
  misc_feature 1..22: note = CHu-sRNA-23
  source 1..22: mol_type = other RNA
taacttatcagactgatgttga

SEQ ID NO: 66 - RNA, 21 nt, synthetic construct
  misc_feature 1..21: note = CHu-sRNA-24
  source 1..21: mol_type = other RNA
tgatgtagtaggttgtatagt

SEQ ID NO: 67 - RNA, 22 nt, synthetic construct
  misc_feature 1..22: note = CHu-sRNA-25
  source 1..22: mol_type = other RNA
tgatgtagtaggttgtatggtt

SEQ ID NO: 68 - RNA, 19 nt, synthetic construct
  misc_feature 1..19: note = CHu-sRNA-26
  source 1..19: mol_type = other RNA
ttaaagtaatccaggatag

SEQ ID NO: 69 - RNA, 22 nt, synthetic construct
  misc_feature 1..22: note = CHu-sRNA-27
  source 1..22: mol_type = other RNA
tgtaaacatcctcgactggaaa

SEQ ID NO: 70 - RNA, 20 nt, synthetic construct
  misc_feature 1..20: note = CHu-sRNA-28
  source 1..20: mol_type = other RNA
ttaaagtaatccaggatagg

SEQ ID NO: 71 - RNA, 20 nt, synthetic construct
  misc_feature 1..20: note = CHu-sRNA-29
  source 1..20: mol_type = other RNA
ttagagtaatccaggatagg

SEQ ID NO: 72 - RNA, 22 nt, synthetic construct
  misc_feature 1..22: note = CHu-sRNA-30
  source 1..22: mol_type = other RNA
tgatgtagtaggttgtatagtt

SEQ ID NO: 73 - RNA, 20 nt, synthetic construct
  misc_feature 1..20: note = CHu-sRNA-31
  source 1..20: mol_type = other RNA
tgctgtagtagattgtatag

SEQ ID NO: 74 - RNA, 20 nt, synthetic construct
  misc_feature 1..20: note = CHu-sRNA-32
  source 1..20: mol_type = other RNA
tccagtactgtgataactga

SEQ ID NO: 75 - RNA, 21 nt, synthetic construct
  misc_feature 1..21: note = CHu-sRNA-33
  source 1..21: mol_type = other RNA
ccttccctttgtacacaccgc

SEQ ID NO: 76 - RNA, 20 nt, synthetic construct
  misc_feature 1..20: note = CHu-sRNA-34
  source 1..20: mol_type = other RNA
tgcggtagtaggttgtatgg

SEQ ID NO: 77 - RNA, 21 nt, synthetic construct
  misc_feature 1..21: note = CHu-sRNA-35
  source 1..21: mol_type = other RNA
tgctgtagtagattgtatagt

SEQ ID NO: 78 - RNA, 20 nt, synthetic construct
  misc_feature 1..20: note = CHu-sRNA-36
  source 1..20: mol_type = other RNA
tgatgtagtaggttgtgtgg

SEQ ID NO: 79 - RNA, 21 nt, synthetic construct
  misc_feature 1..21: note = CHu-sRNA-37
  source 1..21: mol_type = other RNA
tgatgtagtaggttgtgtggt

SEQ ID NO: 80 - RNA, 21 nt, synthetic construct
  misc_feature 1..21: note = CHu-sRNA-38
  source 1..21: mol_type = other RNA
ttagagtaatccaggataggc

SEQ ID NO: 81 - RNA, 21 nt, synthetic construct
  misc_feature 1..21: note = CHu-sRNA-39
  source 1..21: mol_type = other RNA
ttaaagtaatccaggataggc

SEQ ID NO: 82 - RNA, 19 nt, synthetic construct
  misc_feature 1..19: note = CHu-sRNA-40
  source 1..19: mol_type = other RNA
agccggacggtggccatgg

SEQ ID NO: 83 - RNA, 22 nt, synthetic construct
  misc_feature 1..22: note = CHu-sRNA-41
  source 1..22: mol_type = other RNA
tgctgtagtagattgtatagtt

SEQ ID NO: 84 - RNA, 19 nt, synthetic construct
  misc_feature 1..19: note = CHu-sRNA-42
  source 1..19: mol_type = other RNA
aacccgttaccattactga

SEQ ID NO: 85 - RNA, 21 nt, synthetic construct
  misc_feature 1..21: note = CHu-sRNA-43
  source 1..21: mol_type = other RNA
aacccgttaccattactgagt

SEQ ID NO: 86 - RNA, 19 nt, synthetic construct
  misc_feature 1..19: note = CHu-sRNA-44
  source 1..19: mol_type = other RNA
gtccagtactgtgataact

SEQ ID NO: 87 - RNA, 22 nt, synthetic construct
  misc_feature 1..22: note = CHu-sRNA-45
  source 1..22: mol_type = other RNA
ttaaagtaatccaggataggct

SEQ ID NO: 88 - RNA, 21 nt, synthetic construct
  misc_feature 1..21: note = CHu-sRNA-46
  source 1..21: mol_type = other RNA
taagttatcagactgatgttg

SEQ ID NO: 89 - RNA, 20 nt, synthetic construct
  misc_feature 1..20: note = CHu-sRNA-47
  source 1..20: mol_type = other RNA
gtccagtactgtgataactg

SEQ ID NO: 90 - RNA, 20 nt, synthetic construct
  misc_feature 1..20: note = CHu-sRNA-48
  source 1..20: mol_type = other RNA
tgctgtagtaggttgtatag

SEQ ID NO: 91 - RNA, 19 nt, synthetic construct
  misc_feature 1..19: note = CHu-sRNA-49
  source 1..19: mol_type = other RNA
tcctgagagggagcctgag

SEQ ID NO: 92 - RNA, 22 nt, synthetic construct
  misc_feature 1..22: note = CHu-sRNA-50
  source 1..22: mol_type = other RNA
gttcagagttctacagtccgac

SEQ ID NO: 93 - RNA, 19 nt, synthetic construct
  misc_feature 1..19: note = CHu-sRNA-51
  source 1..19: mol_type = other RNA
tcccggatagctcagtcgg

SEQ ID NO: 94 - RNA, 21 nt, synthetic construct
  misc_feature 1..21: note = CHu-sRNA-52
  source 1..21: mol_type = other RNA
gagcttatcagactgatgttg

SEQ ID NO: 95 - RNA, 22 nt, synthetic construct
  misc_feature 1..22: note = CHu-sRNA-53
  source 1..22: mol_type = other RNA
gagcttatcagactgatgttga

SEQ ID NO: 96 - RNA, 19 nt, synthetic construct
  misc_feature 1..19: note = CHu-sRNA-54
  source 1..19: mol_type = other RNA
tcactccgaagtttccctc

SEQ ID NO: 97 - RNA, 21 nt, synthetic construct
  misc_feature 1..21: note = CHu-sRNA-55
  source 1..21: mol_type = other RNA
tttcagagttctacagtccga

SEQ ID NO: 98 - RNA, 19 nt, synthetic construct
  misc_feature 1..19: note = DDi-sRNA-1
  source 1..19: mol_type = other RNA
tgatatgaagcactgtagc

SEQ ID NO: 99 - RNA, 22 nt, synthetic construct
  misc_feature 1..22: note = HQi-sRNA-1
  source 1..22: mol_type = other RNA
ccctgcccttgtacacaccgcc

SEQ ID NO: 100 - RNA, 21 nt, synthetic construct
  misc_feature 1..21: note = HQi-sRNA-2
  source 1..21: mol_type = other RNA
atggttcgattccggagaggg

SEQ ID NO: 101 - RNA, 24 nt, synthetic construct
  misc_feature 1..24: note = JYH-sRNA-1
  source 1..24: mol_type = other RNA
ttcagagttctacagtccgacgat

SEQ ID NO: 102 - RNA, 18 nt, synthetic construct
  misc_feature 1..18: note = LQi-sRNA-1
  source 1..18: mol_type = other RNA
gcctgtctgagcgtcgtt

SEQ ID NO: 103 - RNA, 18 nt, synthetic construct
  misc_feature 1..18: note = LQi-sRNA-2
  source 1..18: mol_type = other RNA
tccctggttgatcctgcc

SEQ ID NO: 104 - RNA, 18 nt, synthetic construct
  misc_feature 1..18: note = LQi-sRNA-3
  source 1..18: mol_type = other RNA
tagtggtatgattctcgc

SEQ ID NO: 105 - RNA, 19 nt, synthetic construct
  misc_feature 1..19: note = LQi-sRNA-4
  source 1..19: mol_type = other RNA
ctttcagcaacggatctct

SEQ ID NO: 106 - RNA, 26 nt, synthetic construct
  misc_feature 1..26: note = LQi-sRNA-5
  source 1..26: mol_type = other RNA
cttcagagttctacagtccgacgatc

SEQ ID NO: 107 - RNA, 18 nt, synthetic construct
  misc_feature 1..18: note = LQi-sRNA-6
  source 1..18: mol_type = other RNA
atcctgctggcgtcgcca

SEQ ID NO: 108 - RNA, 21 nt, synthetic construct
  misc_feature 1..21: note = LQi-sRNA-7
  source 1..21: mol_type = other RNA
atccacggccataggactttg

SEQ ID NO: 109 - RNA, 21 nt, synthetic construct
  misc_feature 1..21: note = LQi-sRNA-8
  source 1..21: mol_type = other RNA
tccatggtctagtggttagga

SEQ ID NO: 110 - RNA, 18 nt, synthetic construct
  misc_feature 1..18: note = XKC-sRNA-1
  source 1..18: mol_type = other RNA
cgctggcaagggccctgg

SEQ ID NO: 111 - RNA, 19 nt, synthetic construct
  misc_feature 1..19: note = XKC-sRNA-2
  source 1..19: mol_type = other RNA
cgctggcaagggccctggg

SEQ ID NO: 112 - RNA, 18 nt, synthetic construct
  misc_feature 1..18: note = CCCCCGGUUCAAUCCCGG
  source 1..18: mol_type = other RNA
cccccggttcaatcccgg

SEQ ID NO: 113 - RNA, 18 nt, synthetic construct
  misc_feature 1..18: note = XKC-sRNA-4
  source 1..18: mol_type = other RNA
cccccggttcagtcccgg

SEQ ID NO: 114 - RNA, 20 nt, synthetic construct
  misc_feature 1..20: note = XKC-sRNA-5
  source 1..20: mol_type = other RNA
tccatggtctagtggttagg

SEQ ID NO: 115 - RNA, 21 nt, synthetic construct
  misc_feature 1..21: note = XKC-sRNA-6
  source 1..21: mol_type = other RNA
cccactgctaaatttgactgg

SEQ ID NO: 116 - RNA, 27 nt, synthetic construct
  misc_feature 1..27: note = XKC-sRNA-7
  source 1..27: mol_type = other RNA
ccggggctacgcctgtctgagcgtcgc

SEQ ID NO: 117 - RNA, 24 nt, synthetic construct
  misc_feature 1..24: note = XKC-sRNA-8
  source 1..24: mol_type = other RNA
ggctacgcctgtctgagcgtcgct

SEQ ID NO: 118 - RNA, 21 nt, synthetic construct
  misc_feature 1..21: note = YXC-sRNA-1
  source 1..21: mol_type = other RNA
ccgcggggccccgtcgtcccc

SEQ ID NO: 119 - RNA, 21 nt, synthetic construct
  misc_feature 1..21: note = YXC-sRNA-2
  source 1..21: mol_type = other RNA
cccgcggggccccgtcgtccc

SEQ ID NO: 120 - RNA, 22 nt, synthetic construct
  misc_feature 1..22: note = YXC-sRNA-3
  source 1..22: mol_type = other RNA
cccgcggggccccgtcgtcccc

SEQ ID NO: 121 - RNA, 22 nt, synthetic construct
  misc_feature 1..22: note = YXC-sRNA-4
  source 1..22: mol_type = other RNA
ccgcggggccccgtcgtccccc

SEQ ID NO: 122 - RNA, 26 nt, synthetic construct
  misc_feature 1..26: note = YXC-sRNA-5
  source 1..26: mol_type = other RNA
tgcaatgatgtcatcttactactgaa

SEQ ID NO: 123 - RNA, 23 nt, synthetic construct
  misc_feature 1..23: note = YXC-sRNA-6
  source 1..23: mol_type = other RNA
cccgcggggccccgtcgtccccc

SEQ ID NO: 124 - RNA, 21 nt, synthetic construct
  misc_feature 1..21: note = YXC-sRNA-7
  source 1..21: mol_type = other RNA
cccagtgtttagactacctgt

SEQ ID NO: 125 - RNA, 23 nt, synthetic construct
  misc_feature 1..23: note = YXC-sRNA-8
  source 1..23: mol_type = other RNA
aggcagtgtagttagctgattga

SEQ ID NO: 126 - RNA, 21 nt, synthetic construct
  misc_feature 1..21: note = YXC-sRNA-9
  source 1..21: mol_type = other RNA
ccagtgtttagactacctgtt

SEQ ID NO: 127 - RNA, 22 nt, synthetic construct
  misc_feature 1..22: note = YXC-sRNA-10
  source 1..22: mol_type = other RNA
cccagtgtttagactacctgtt

SEQ ID NO: 128 - RNA, 21 nt, synthetic construct
  misc_feature 1..21: note = YXC-sRNA-11
  source 1..21: mol_type = other RNA
taatactgtctggtaatgccg

SEQ ID NO: 129 - RNA, 19 nt, synthetic construct
  misc_feature 1..19: note = YXC-sRNA-12
  source 1..19: mol_type = other RNA
tgtagtaggttgtatagtt

SEQ ID NO: 130 - RNA, 19 nt, synthetic construct
  misc_feature 1..19: note = YXC-sRNA-13
  source 1..19: mol_type = other RNA
tgtagtaggttgtatggtt

SEQ ID NO: 131 - RNA, 22 nt, synthetic construct
  misc_feature 1..22: note = YXC-sRNA-14
  source 1..22: mol_type = other RNA
taatactgtctggtaatgccgt

SEQ ID NO: 132 - RNA, 19 nt, synthetic construct
  misc_feature 1..19: note = YXC-sRNA-15
  source 1..19: mol_type = other RNA
tgatgtagtaggttgtata

SEQ ID NO: 133 - RNA, 23 nt, synthetic construct
  misc_feature 1..23: note = YXC-sRNA-16
  source 1..23: mol_type = other RNA
tgtaaacatcctcgactggaaga

SEQ ID NO: 134 - RNA, 23 nt, synthetic construct
  misc_feature 1..23: note = YXC-sRNA-17
  source 1..23: mol_type = other RNA
cagcagcaattcatgttttggaa

SEQ ID NO: 135 - RNA, 22 nt, synthetic construct
  misc_feature 1..22: note = YXC-sRNA-18
  source 1..22: mol_type = other RNA
ccagtgtttagactacctgttc

SEQ ID NO: 136 - RNA, 23 nt, synthetic construct
  misc_feature 1..23: note = YXC-sRNA-19
  source 1..23: mol_type = other RNA
cccagtgtttagactacctgttc

SEQ ID NO: 137 - RNA, 23 nt, synthetic construct
  misc_feature 1..23: note = YXC-sRNA-20
  source 1..23: mol_type = other RNA
ccccgcggggccccgtcgtcccc

SEQ ID NO: 138 - RNA, 20 nt, synthetic construct
  misc_feature 1..20: note = YXC-sRNA-21
  source 1..20: mol_type = other RNA
tccctgaggagccctttgag

SEQ ID NO: 139 - RNA, 19 nt, synthetic construct
  misc_feature 1..19: note = YXC-sRNA-22
  source 1..19: mol_type = other RNA
tgctgtagtagattgtata

SEQ ID NO: 140 - RNA, 21 nt, synthetic construct
  misc_feature 1..21: note = YXC-sRNA-23
  source 1..21: mol_type = other RNA
aaggttacttgttagttcagg

SEQ ID NO: 141 - RNA, 24 nt, synthetic construct
  misc_feature 1..24: note = YXC-sRNA-24
  source 1..24: mol_type = other RNA
ccccgcggggccccgtcgtccccc

SEQ ID NO: 142 - RNA, 19 nt, synthetic construct
  misc_feature 1..19: note = YXC-sRNA-25
  source 1..19: mol_type = other RNA
tgtagtaggttgtgtggtt

SEQ ID NO: 143 - RNA, 21 nt, synthetic construct
  misc_feature 1..21: note = YXC-sRNA-26
  source 1..21: mol_type = other RNA
ttaatgctaattgtgataggg

SEQ ID NO: 144 - RNA, 19 nt, synthetic construct
  misc_feature 1..19: note = YXC-sRNA-27
  source 1..19: mol_type = other RNA
tgatgtagtagtttgtaca

SEQ ID NO: 145 - RNA, 20 nt, synthetic construct
  misc_feature 1..20: note = YXC-sRNA-28
  source 1..20: mol_type = other RNA
tgatgtagtagtttgtacag

SEQ ID NO: 146 - RNA, 22 nt, synthetic construct
  misc_feature 1..22: note = YXC-sRNA-29
  source 1..22: mol_type = other RNA
tgatgtagtaggttgtgtggtt

SEQ ID NO: 147 - RNA, 21 nt, synthetic construct
  misc_feature 1..21: note = YXC-sRNA-30
  source 1..21: mol_type = other RNA
tgatgtagtagtttgtacagt

SEQ ID NO: 148 - RNA, 21 nt, synthetic construct
  misc_feature 1..21: note = YXC-sRNA-31
  source 1..21: mol_type = other RNA
tgctgtagtaggttgtatagt

SEQ ID NO: 149 - RNA, 22 nt, synthetic construct
  misc_feature 1..22: note = YXC-sRNA-32
  source 1..22: mol_type = other RNA
tgatgtagtagtttgtacagtt

SEQ ID NO: 150 - RNA, 22 nt, synthetic construct
  misc_feature 1..22: note = YXC-sRNA-33
  source 1..22: mol_type = other RNA
tccctgaggagccctttgagcc

SEQ ID NO: 151 - RNA, 20 nt, synthetic construct
  misc_feature 1..20: note = YXC-sRNA-34
  source 1..20: mol_type = other RNA
tgctgtagtaggttgtatgg

SEQ ID NO: 152 - RNA, 21 nt, synthetic construct
  misc_feature 1..21: note = YXC-sRNA-35
  source 1..21: mol_type = other RNA
tgctgtagtaggttgtatggt

SEQ ID NO: 153 - RNA, 20 nt, synthetic construct
  misc_feature 1..20: note = YXC-sRNA-36
  source 1..20: mol_type = other RNA
aacccgttaccattactgag

SEQ ID NO: 154 - RNA, 19 nt, synthetic construct
  misc_feature 1..19: note = YXC-sRNA-37
  source 1..19: mol_type = other RNA
tgctgtagtagtttgtgct

SEQ ID NO: 155 - RNA, 22 nt, synthetic construct
  misc_feature 1..22: note = YXC-sRNA-38
  source 1..22: mol_type = other RNA
tgctgtagtaggttgtatagtt

SEQ ID NO: 156 - RNA, 21 nt, synthetic construct
  misc_feature 1..21: note = YXC-sRNA-39
  source 1..21: mol_type = other RNA
tgctgtagtagtttgtgctgt

SEQ ID NO: 157 - RNA, 22 nt, synthetic construct
  misc_feature 1..22: note = YXC-sRNA-40
  source 1..22: mol_type = other RNA
tgctgtagtagtttgtgctgtt

SEQ ID NO: 158 - RNA, 19 nt, synthetic construct
  misc_feature 1..19: note = YXC-sRNA-41
  source 1..19: mol_type = other RNA
tgtgaacatcctcgactgg

SEQ ID NO: 159 - RNA, 20 nt, synthetic construct
  misc_feature 1..20: note = YXC-sRNA-42
  source 1..20: mol_type = other RNA
tgtgaacatcctcgactgga

SEQ ID NO: 160 - RNA, 22 nt, synthetic construct
  misc_feature 1..22: note = YXC-sRNA-43
  source 1..22: mol_type = other RNA
tgctgtagtaggttgtatggtt

SEQ ID NO: 161 - RNA, 24 nt, synthetic construct
  misc_feature 1..24: note = YXC-sRNA-44
  source 1..24: mol_type = other RNA
taatactgcctggtaatgatgact

SEQ ID NO: 162 - RNA, 21 nt, synthetic construct
  misc_feature 1..21: note = YXC-sRNA-45
  source 1..21: mol_type = other RNA
tgtgaacatcctcgactggaa

SEQ ID NO: 163 - RNA, 21 nt, synthetic construct
  misc_feature 1..21: note = YXC-sRNA-46
  source 1..21: mol_type = other RNA
gtccagtactgtgataactga

SEQ ID NO: 164 - RNA, 22 nt, synthetic construct
  misc_feature 1..22: note = YXC-sRNA-47
  source 1..22: mol_type = other RNA
aacccgttaccattactgagtt

SEQ ID NO: 165 - RNA, 21 nt, synthetic construct
  misc_feature 1..21: note = YXC-sRNA-48
  source 1..21: mol_type = other RNA
agatgtagtaggttgcatagt

SEQ ID NO: 166 - RNA, 21 nt, synthetic construct
  misc_feature 1..21: note = YXC-sRNA-49
  source 1..21: mol_type = other RNA
agggttcgagtgtgagcatgc

SEQ ID NO: 167 - RNA, 18 nt, synthetic construct
  misc_feature 1..18: note = YXC-sRNA-50
  source 1..18: mol_type = other RNA
tgatatgaagcactgtag

SEQ ID NO: 168 - RNA, 19 nt, synthetic construct
  misc_feature 1..19: note = YXC-sRNA-51
  source 1..19: mol_type = other RNA
aacccgtcctcagttcgga

SEQ ID NO: 169 - RNA, 18 nt, synthetic construct
  misc_feature 1..18: note = YXC-sRNA-52
  source 1..18: mol_type = other RNA
tgctatgaagcactgtag

SEQ ID NO: 170 - RNA, 19 nt, synthetic construct
  misc_feature 1..19: note = YXC-sRNA-53
  source 1..19: mol_type = other RNA
tgctatgaagcactgtagc

SEQ ID NO: 171 - RNA, 20 nt, synthetic construct
  misc_feature 1..20: note = YXC-sRNA-54
  source 1..20: mol_type = other RNA
tgctatgaagcactgtagct

SEQ ID NO: 172 - RNA, 18 nt, synthetic construct
  misc_feature 1..18: note = YXC-sRNA-55
  source 1..18: mol_type = other RNA
tgatgtagtagattgtat

SEQ ID NO: 173 - RNA, 21 nt, synthetic construct
  misc_feature 1..21: note = YXC-sRNA-56
  source 1..21: mol_type = other RNA
tgctatgaagcactgtagctc

SEQ ID NO: 174 - RNA, 23 nt, synthetic construct
  misc_feature 1..23: note = YXC-sRNA-57
  source 1..23: mol_type = other RNA
tcgatcctggctcaggatgaacg

SEQ ID NO: 175 - RNA, 22 nt, synthetic construct
  misc_feature 1..22: note = YXC-sRNA-58
  source 1..22: mol_type = other RNA
tgctatgaagcactgtagctct

SEQ ID NO: 176 - RNA, 19 nt, synthetic construct
  misc_feature 1..19: note = YXC-sRNA-59
  source 1..19: mol_type = other RNA
tgatgtagtagtttgtgct

SEQ ID NO: 177 - RNA, 20 nt, synthetic construct
  misc_feature 1..20: note = YXC-sRNA-60
  source 1..20: mol_type = other RNA
tgatgtagtagtttgtgctg

SEQ ID NO: 178 - RNA, 21 nt, synthetic construct
  misc_feature 1..21: note = YXC-sRNA-61
  source 1..21: mol_type = other RNA
tgatgtagtagtttgtgctgt

SEQ ID NO: 179 - RNA, 21 nt, synthetic construct
  misc_feature 1..21: note = YXC-sRNA-62
  source 1..21: mol_type = other RNA
tcttcccagtgctctgaatgt

SEQ ID NO: 180 - RNA, 22 nt, synthetic construct
  misc_feature 1..22: note = YXC-sRNA-63
  source 1..22: mol_type = other RNA
tgatgtagtagtttgtgctgtt

SEQ ID NO: 181 - RNA, 20 nt, synthetic construct
  misc_feature 1..20: note = YXC-sRNA-64
  source 1..20: mol_type = other RNA
agacacggcccagactccta

SEQ ID NO: 182 - RNA, 18 nt, synthetic construct
  misc_feature 1..18: note = YXC-sRNA-65
  source 1..18: mol_type = other RNA
tgatgtagtaggttgtgt

SEQ ID NO: 183 - RNA, 20 nt, synthetic construct
  misc_feature 1..20: note = YXC-sRNA-66
  source 1..20: mol_type = other RNA
gtattgtttcctactttatg

SEQ ID NO: 184 - RNA, 21 nt, synthetic construct
  misc_feature 1..21: note = YXC-sRNA-67
  source 1..21: mol_type = other RNA
gtattgtttcctactttatgg

SEQ ID NO: 185 - RNA, 22 nt, synthetic construct
  misc_feature 1..22: note = YXC-sRNA-68
  source 1..22: mol_type = other RNA
gtattgtttcctactttatgga

SEQ ID NO: 186 - RNA, 20 nt, synthetic construct
  misc_feature 1..20: note = YXC-sRNA-69
  source 1..20: mol_type = other RNA
tggaaacatcctcgactgga

SEQ ID NO: 187 - RNA, 20 nt, synthetic construct
  misc_feature 1..20: note = YXC-sRNA-70
  source 1..20: mol_type = other RNA
acattagtctgcacattggt

SEQ ID NO: 188 - RNA, 21 nt, synthetic construct
  misc_feature 1..21: note = YXC-sRNA-71
  source 1..21: mol_type = other RNA
tggaaacatcctcgactggaa

SEQ ID NO: 189 - RNA, 21 nt, synthetic construct
  misc_feature 1..21: note = YXC-sRNA-72
  source 1..21: mol_type = other RNA
atcttatcagactgatgttga

SEQ ID NO: 190 - RNA, 21 nt, synthetic construct
  misc_feature 1..21: note = YXC-sRNA-73
  source 1..21: mol_type = other RNA
acattagtctgcacattggtt

SEQ ID NO: 191 - RNA, 19 nt, synthetic construct
  misc_feature 1..19: note = YXC-sRNA-74
  source 1..19: mol_type = other RNA
tgttcaaatccatgcaaaa

SEQ ID NO: 192 - RNA, 19 nt, synthetic construct
  misc_feature 1..19: note = YXC-sRNA-75
  source 1..19: mol_type = other RNA
tcttaccgtgagtaataat

SEQ ID NO: 193 - RNA, 22 nt, synthetic construct
  misc_feature 1..22: note = YXC-sRNA-76
  source 1..22: mol_type = other RNA
tatcttatcagactgatgttga

SEQ ID NO: 194 - RNA, 20 nt, synthetic construct
  misc_feature 1..20: note = YXC-sRNA-77
  source 1..20: mol_type = other RNA
tcttaccgtgagtaataatg

SEQ ID NO: 195 - RNA, 22 nt, synthetic construct
  misc_feature 1..22: note = YXC-sRNA-78
  source 1..22: mol_type = other RNA
tgttcaaatccatgcaaaactg

SEQ ID NO: 196 - RNA, 20 nt, synthetic construct
  misc_feature 1..20: note = YXC-sRNA-79
  source 1..20: mol_type = other RNA
tatcaccatctgaaatcggt

SEQ ID NO: 197 - RNA, 23 nt, synthetic construct
  misc_feature 1..23: note = YXC-sRNA-80
  source 1..23: mol_type = other RNA
tgttcaaatccatgcaaaactga

SEQ ID NO: 198 - RNA, 20 nt, synthetic construct
  misc_feature 1..20: note = YXC-sRNA-81
  source 1..20: mol_type = other RNA
tcataccgtgagtaataatg

SEQ ID NO: 199 - RNA, 21 nt, synthetic construct
  misc_feature 1..21: note = YXC-sRNA-82
  source 1..21: mol_type = other RNA
tatcaccatctgaaatcggtt

SEQ ID NO: 200 - RNA, 22 nt, synthetic construct
  misc_feature 1..22: note = YXC-sRNA-83
  source 1..22: mol_type = other RNA
tgatatgaagcactgtagctca

SEQ ID NO: 201 - RNA, 33 nt, synthetic construct
  misc_feature 1..33: note = CXL-sRNA-30
  source 1..33: mol_type = other RNA
gggattgtagttcaattggtcagagcaccgccc

SEQ ID NO: 202 - RNA, 19 nt, synthetic construct
  misc_feature 1..19: note = PGY-sRNA-21
  source 1..19: mol_type = other RNA
gtgcttgaaattgtcggga

SEQ ID NO: 203 - RNA, 21 nt, synthetic construct
  misc_feature 1..21: note = PGY-sRNA-22
  source 1..21: mol_type = other RNA
tgaactctgaactccagtcac

SEQ ID NO: 204 - RNA, 19 nt, synthetic construct
  misc_feature 1..19: note = PGY-sRNA-23
  source 1..19: mol_type = other RNA
ccctccgcggccagcttct

SEQ ID NO: 205 - RNA, 18 nt, synthetic construct
  misc_feature 1..18: note = PGY-sRNA-24
  source 1..18: mol_type = other RNA
gtgtcgtgagatgttggg

SEQ ID NO: 206 - RNA, 28 nt, synthetic construct
  misc_feature 1..28: note = PGY-sRNA-25
  source 1..28: mol_type = other RNA
gttcagagttctacagtccgacgatctc

SEQ ID NO: 207 - RNA, 25 nt, synthetic construct
  misc_feature 1..25: note = PGY-sRNA-26
  source 1..25: mol_type = other RNA
tccggaatgattgggcgtaaagcgt

SEQ ID NO: 208 - RNA, 19 nt, synthetic construct
  misc_feature 1..19: note = PGY-sRNA-27
  source 1..19: mol_type = other RNA
accgtgcgctggattatga

SEQ ID NO: 209 - RNA, 24 nt, synthetic construct
  misc_feature 1..24: note = PGY-sRNA-28
  source 1..24: mol_type = other RNA
tctcaggtagacagtttctatggg

SEQ ID NO: 210 - RNA, 22 nt, synthetic construct
  misc_feature 1..22: note = PGY-sRNA-29
  source 1..22: mol_type = other RNA
cgatcctggctcaggatgaacg

SEQ ID NO: 211 - RNA, 21 nt, synthetic construct
  misc_feature 1..21: note = PGY-sRNA-30
  source 1..21: mol_type = other RNA
tttggattgaagggagctctg

SEQ ID NO: 212 - RNA, 19 nt, synthetic construct
  misc_feature 1..19: note = PGY-sRNA-31
  source 1..19: mol_type = other RNA
agcttaccaaggcgatgat

SEQ ID NO: 213 - RNA, 20 nt, synthetic construct
  misc_feature 1..20: note = PGY-sRNA-32
  source 1..20: mol_type = other RNA
ccggccccgaacccgtcggc

SEQ ID NO: 214 - RNA, 21 nt, synthetic construct
  misc_feature 1..21: note = PGY-sRNA-6
  source 1..21: mol_type = other RNA
gttcagagttctacagtccga

SEQ ID NO: 215 - RNA, 26 nt, synthetic construct
  misc_feature 1..26: note = PGY-sRNA-18
  source 1..26: mol_type = other RNA
cggggctacgcctgtctgagcgtcgc

SEQ ID NO: 216 - RNA, 21 nt, synthetic construct
  misc_feature 1..21: note = sly-miR168b-5p
  source 1..21: mol_type = other RNA
tcgcttggtgcaggtcgggac

SEQ ID NO: 217 - RNA, 19 nt, synthetic construct
  misc_feature 1..19: note = Pab-miR3711
  source 1..19: mol_type = other RNA
ggccctccttctagcgcca

SEQ ID NO: 218 - RNA, 18 nt, synthetic construct
  misc_feature 1..18: note = CXL-sRNA-17
  source 1..18: mol_type = other RNA
cagagtcgcgcagcggaa

SEQ ID NO: 219 - RNA, 24 nt, synthetic construct
  misc_feature 1..24: note = CXL-sRNA-21
  source 1..24: mol_type = other RNA
acagcaggacggtggccatggaag

SEQ ID NO: 220 - RNA, 21 nt, synthetic construct
  misc_feature 1..21: note = ppe-miR169c
  source 1..21: mol_type = other RNA
cagccaaggatgacttgccgg

SEQ ID NO: 221 - RNA, 21 nt, synthetic construct
  misc_feature 1..21: note = HJT-sRNA-a2
  source 1..21: mol_type = other RNA
tagcaccatccgaaatcggta

SEQ ID NO: 222 - RNA, 27 nt, synthetic construct
  misc_feature 1..27: note = HJT-sRNA-h3
  source 1..27: mol_type = other RNA
tggggctacgcctgtctgagcgtcgct

SEQ ID NO: 223 - DNA, 21 bp, synthetic construct
  misc_feature 1..21: note = random nonsense sequence: uucuccgaacgugucacgutt
  source 1..21: mol_type = other DNA
ttctccgaacgtgtcacgttt

SEQ ID NO: 224 - DNA, 21 bp, synthetic construct
  misc_feature 1..21: note = primer
  source 1..21: mol_type = other DNA
ctggaagatggtcgtaccctg

SEQ ID NO: 225 - DNA, 20 bp, synthetic construct
  misc_feature 1..20: note = primer
  source 1..20: mol_type = other DNA
ggtcttgccagtgagtgtct

SEQ ID NO: 226 - DNA, 21 bp, synthetic construct
  misc_feature 1..21: note = primer
  source 1..21: mol_type = other DNA
ctcgccagtgaaatgatggct

SEQ ID NO: 227 - DNA, 21 bp, synthetic construct
  misc_feature 1..21: note = primer
  source 1..21: mol_type = other DNA
gtcggagattcgtagctggat

SEQ ID NO: 228 - DNA, 21 bp, synthetic construct
  misc_feature 1..21: note = primer
  source 1..21: mol_type = other DNA
ggtacatcctcgacggcatct

SEQ ID NO: 229 - DNA, 21 bp, synthetic construct
  misc_feature 1..21: note = primer
  source 1..21: mol_type = other DNA
gtgcctctttgctgctttcac

SEQ ID NO: 230 - DNA, 19 bp, synthetic construct
  misc_feature 1..19: note = primer
  source 1..19: mol_type = other DNA
ctgccccaatccctttatt

SEQ ID NO: 231 - DNA, 20 bp, synthetic construct
  misc_feature 1..20: note = primer
  source 1..20: mol_type = other DNA
cccaattctctttttgagcc

SEQ ID NO: 232 - DNA, 19 bp, synthetic construct
  misc_feature 1..19: note = primer
  source 1..19: mol_type = other DNA
gttcccattagacaactgc

SEQ ID NO: 233 - DNA, 18 bp, synthetic construct
  misc_feature 1..18: note = primer
  source 1..18: mol_type = other DNA
gattctttcctttgaggc

SEQ ID NO: 234 - DNA, 23 bp, synthetic construct
  misc_feature 1..23: note = primer
  source 1..23: mol_type = other DNA
tagtccttcctaccccaatttcc

SEQ ID NO: 235 - DNA, 21 bp, synthetic construct
  misc_feature 1..21: note = primer
  source 1..21: mol_type = other DNA
ttggtccttagccactccttc

SEQ ID NO: 236 - DNA, 19 bp, synthetic construct
  misc_feature 1..19: note = primer
  source 1..19: mol_type = other DNA
cctgtagcccacgtcgtag

SEQ ID NO: 237 - DNA, 22 bp, synthetic construct
  misc_feature 1..22: note = primer
  source 1..22: mol_type = other DNA
gggagtagacaaggtacaaccc

SEQ ID NO: 238 - DNA, 24 bp, synthetic construct
  misc_feature 1..24: note = primer
  source 1..24: mol_type = other DNA
cactcacggcaaattcaacggcac

SEQ ID NO: 239 - DNA, 22 bp, synthetic construct
  misc_feature 1..22: note = primer
  source 1..22: mol_type = other DNA
gactccacgacatactcagcac